European Patent Application EP 4 707 295 A1, published March 11, 2026. Title: INTERLEUKIN-2 VARIANTS WITH MODIFIED BIOLOGICAL ACTIVITY. Applicant: EGLE THERAPEUTICS. Application EP. The sequence listing filed with the application follows.

SEQUENCE LISTING (14 sequences)

SEQ ID NO: 1 - protein, 133 aa, Homo sapiens [sequence omitted]

SEQ ID NO: 2 - protein, 132 aa, synthetic construct
APTSSTKETQEQLEHLLRDLQLILKGINNPKNPKLTRMLTFKFYMPKQATSLKHLQCLEEELKPLEEVLNLAQSKNFHLEPRNLINNINKIVLKLKGSETTFMCEYADETATIVEFLNRWITFCQSIISRST

SEQ ID NO: 3 - protein, 132 aa, synthetic construct
APTSSTKETQEQLERLLLDLQLILKGINNPKNPKLTRMLTFKFYMPKQATSLKHLQCLEEELKPLEEVLNLAQSKNFHLEPRNLINNINKIVLKLKGSETTFMCEYADETATIVEFLNRWITFCQSIISRST

SEQ ID NO: 4 - protein, 132 aa, synthetic construct
APTSSTKETQEQLERLLRDLQLILKGINNPKNPKLTRMLTFKFYMPKQATSLKHLQCLEEELKPLEEVLNLAQSKNFHLEPRNLINNINVIVLKLKGSETTFMCEYADETATIVEFLNRWITFCQSIISRST

SEQ ID NO: 5 - protein, 132 aa, synthetic construct
APTSSTKETQEQLEHLLLDLQLILKGINNPKNPKLTRMLTFKFYMPKQATSLKHLQCLEEELKPLEEVLNLAQSKNFHLEPRNLINNINKIVLKLKGSETTFMCEYADETATIVEFLNRWITFCQSIISRST

SEQ ID NO: 6 - protein, 132 aa, synthetic construct
APTSSTKETQEQLEHLLRDLQLILKGINNPKNPKLTRMLTFKFYMPKQATSLKHLQCLEEELKPLEEVLNLAQSKNFHLEPRNLINNINVIVLKLKGSETTFMCEYADETATIVEFLNRWITFCQSIISRST

SEQ ID NO: 7 - protein, 132 aa, synthetic construct
APTSSTKETQEQLERLLLDLQLILKGINNPKNPKLTRMLTFKFYMPKQATSLKHLQCLEEELKPLEEVLNLAQSKNFHLEPRNLINNINVIVLKLKGSETTFMCEYADETATIVEFLNRWITFCQSIISRST

SEQ ID NO: 8 - protein, 15 aa, synthetic construct
GGGGSGGGGSGGGGS

SEQ ID NO: 9 - DNA, 396 bp, synthetic construct
  source 1..396: mol_type = other DNA
gccccgaccagcagcactaaagaaacacaggagcaactggagcacctgctgcgcgacctgcaactcatccttaagggtataaataatcctaaaaaccctaagctgacacgcatgcttaccttcaaattctatatgcccaagcaggccacaagcctcaagcacctgcaatgtcttgaagaagaattgaagcccctggaggaggtgcttaacctggcgcagtctaagaattttcacctggagccgcggaacctgataaacaatatcaacaaaatagtcctcaaactgaagggcagcgaaactacattcatgtgtgaatacgcagatgaaacggctactatagtcgagtttctaaatcggtggattaccttttgccagtccattataagccggagcact

SEQ ID NO: 10 - DNA, 396 bp, synthetic construct
  source 1..396: mol_type = other DNA
gccccgacctctagcactaaggagactcaggagcagttggagaggctacttcttgatctgcaactgatcctgaagggcattaacaaccccaagaacccaaagctcacgaggatgctgacttttaagttctatatgcctaaacaagcaactagtttaaaacatctgcaatgtttggaggaggagttaaagcctctggaggaggtgctcaacttggcccaaagcaagaactttcacctagaaccgcggaacctgattaataatatcaacaagatagtcctgaaactcaaaggatcggaaacgacattcatgtgcgagtacgcagacgaaaccgcaaccatagtcgagtttctgaatcgttggataacattttgccagagcattatcagtcggtcaaca

SEQ ID NO: 11 - DNA, 396 bp, synthetic construct
  source 1..396: mol_type = other DNA
gccccaaccagtagcacgaaggaaacacaagaacaacttgaacggctcctgagggacctgcaactgatcctaaaaggaattaacaaccccaagaatccaaagctgacgcgcatgctcacattcaagttttatatgcctaagcaagctactagcctcaagcatctgcaatgtctggaggaagagttgaagccattagaggaagtcctcaatctggcacaatcaaaaaatttccacttggagccgcggaacttgataaataatatcaatgtgatagtcctgaaactaaaaggttctgaaactacatttatgtgtgagtacgccgacgagaccgcaacaatagtcgagttcctaaaccgctggattaccttttgtcaaagtataatctcgcgaagcact

SEQ ID NO: 12 - DNA, 396 bp, synthetic construct
  source 1..396: mol_type = other DNA
gccccgaccagcagcactaaagaaacacaggagcaactggagcacctgctgttagacctgcaactcatccttaagggtataaataatcctaaaaaccctaagctgacacgcatgctcacgttcaaattctatatgcccaagcaggccacaagcctcaagcacctgcaatgtcttgaagaagaattgaagcccctggaggaggtgcttaacctggcgcagtctaagaattttcacctggagccgcggaacctgataaataatatcaacaaaatagtcctcaaactgaagggctcggaaactacattcatgtgtgaatacgcagatgaaacggctactatagtcgagtttctaaatcggtggattaccttttgccagtccattataagccggagcact

SEQ ID NO: 13 - DNA, 396 bp, synthetic construct
  source 1..396: mol_type = other DNA
gccccaacaagctcaactaaagagacccaagagcaactggaacacttgttgcgcgacctgcaactgattcttaaaggcatcaacaatcctaagaatcccaaactgacccgcatgctgaccttcaaattttacatgccaaaacaagccacttctctgaaacacctgcaatgtcttgaagaggagctgaagcccctggaggaagtcttgaacctggctcaaagcaagaactttcatctggagccgcggaacttgatcaacaacatcaatgtgatagtccttaaactcaaggggagtgagacgacatttatgtgcgagtacgccgatgagaccgcaactatagtcgagttcctgaatagatggataactttttgccaatcaatcataagccgatcaacc

SEQ ID NO: 14 - DNA, 396 bp, synthetic construct
  source 1..396: mol_type = other DNA
gcaccgacatcttcaacaaaggaaacacaggagcagttggagaggttactgcttgacctgcaactcatcttgaaagggatcaataaccctaagaaccccaagttgaccagaatgttgacgttcaagttttatatgccgaagcaggctaccagcttgaagcacctgcaatgtctggaggaggagcttaaaccactggaggaggtcttgaatctagcgcagtcaaaaaactttcatttggaaccgcggaacttgattaacaacataaacgtcatagtcctcaagctgaaaggcagcgaaaccacgtttatgtgcgaatacgcagatgaaacagctacaatagtcgagttcttgaacaggtggatcacattttgccagtctatcatatcgcggtctacg